European Patent Application EP 4 378 319 A1, published June 5, 2024. Title: COMPOSITION COMPRISING BIOACTIVE PEPTIDES. Applicant: Bioiberica S.A.U. The sequence listing filed with the application follows.

SEQUENCE LISTING (7 sequences)

SEQ ID NO: 1 - protein, 14 aa, synthetic construct
  source 1..14: note = Peptide obtained by enzymatic hydrolisis of porcine mucosa; note (original language) = peptido obtenido por hidrolisis enzimatica de mucosa porcina; organism (original language) = construccion sintetica
TNVPRASVPDGFLS

SEQ ID NO: 2 - protein, 16 aa, synthetic construct
  source 1..16: note = Peptide obtained by enzymatic hydrolisis of porcine mucosa; note (original language) = peptido obtenido por hidrolisis enzimatica de mucosa porcina; organism (original language) = contruccion sintetica
TNVPRASVPDGFLSEL

SEQ ID NO: 3 - protein, 11 aa, synthetic construct
  source 1..11: note = Peptide obtained by enzymatic hydrolisis of porcine mucosa; note (original language) = peptido obtenido por hidrolisis enzimatica de mucosa porcina; organism (original language) = construccion sintetica
DAVEDLESVGK

SEQ ID NO: 4 - protein, 15 aa, synthetic construct
  source 1..15: note = Peptide obtained by enzymatic hydrolisis of porcine mucosa; note (original language) = peptido obtenido por hidrolisis enzimatica de mucosa porcina; organism (original language) = contruccion sintetica
EGIPPDQQRLIFAGK

SEQ ID NO: 5 - protein, 16 aa, synthetic construct
  source 1..16: note = Peptide obtained by enzymatic hydrolisis of porcine mucosa; note (original language) = peptido obtenido por hidrolisis enzimatica de mucosa porcina; organism (original language) = construccion sintetica
TITLEVEPSDTIENVK

SEQ ID NO: 6 - protein, 11 aa, synthetic construct
  source 1..11: note = Peptide obtained by enzymatic hydrolisis of porcine mucosa; note (original language) = peptido obtenido por hidrolisis enzimatica de mucosa porcina; organism (original language) = construccion sintetica
VHVVPDQLMAF

SEQ ID NO: 7 - protein, 14 aa, synthetic construct
  source 1..14: note = Peptide obtained by enzymatic hydrolisis of porcine mucosa; note (original language) = peptido obtenido por hidrolisis enzimatica de mucosa porcina; organism (original language) = contruccion sintetica
DKEGIPPDQQRLIF